European Patent Specification EP 3 511 417 B1, published May 31, 2023. Title: RIFT VALLEY FEVER VIRUS GLYCOPROTEINS, GN AND GC, AND THEIR USE. Applicant: KANSAS STATE UNIVERSITY RESEARCH FOUNDATION. The sequence listing filed with the application follows.

SEQUENCE LISTING (21 sequences)

SEQ ID NO: 1 - DNA, 54 bp, Rift Valley fever virus
  sig_peptide (1)..(54)
atgacagtccttccagccttagcagtttttgctttggcacctgttgtttttgct

SEQ ID NO: 2 - protein, 18 aa, Rift Valley fever virus
  signal (1)..(18)
MTVLPALAVFALAPVVFA

SEQ ID NO: 3 - DNA, 1354 bp, Rift Valley fever virus
  Kozak (1)..(4)
  sig_peptide (5)..(58)
caccatgacagtccttccagccttagcagtttttgctttggcacctgttgtttttgctgaagacccccatctcagaaacagaccagggaaggggcacaactacattgacgggatgactcaggaggatgccacatgcaaacctgtgacatatgctggggcatgtagcagttttgatgtcttgcttgaaaagggaaaatttccccttttccagtcgtatgctcatcatagaactctactagaggcagttcacgacaccatcattgcaaaggctgatccacctagctgtgaccttctgagtgctcatgggaacccctgcatgaaagagaaactcgtgatgaagacacactgtccaaatgactaccagtcagctcattacctcaacaatgacgggaaaatggcttcagtcaagtgccctcctaagtatgagctcactgaggactgcaacttttgtaggcagatgacaggtgctagcctgaagaaggggtcttatcctctccaagacttgttttgtcagtcaagtgaggatgatggatcaaaattaaaaacaaaaatgaaaggggtctgcgaagtgggggttcaagcactcaaaaagtgtgatggccaactcagcactgcacatgaggttgtgccctttgcagtgtttaagaactcaaagaaggtttatcttgataagcttgaccttaagactgaggagaatctgctaccagactcatttgtctgtttcgagcataagggacagtacaaaggaacaatggactctggtcagactaagagggagctcaaaagctttgatatctctcagtgccccaagattggaggacatggtagtaagaagtgcactggggacgcagcattttgctctgcttatgagtgcactgctcagtacgccaatgcctattgttcacatgctaatgggtcagggattgtgcagatacaagtatcaggggtctggaagaagcctttatgtgtagggtatgagagagtggttgtgaagagagaactctctgccaagcccatccagagagttgagccttgcacaacttgtataaccaaatgtgagcctcatggattggttgtccgatcaacagggttcaagatatcatcagcagttgcttgtgctagcggagtttgcgtcacaggatcgcagagtccttccaccgagattacactcaagtatccagggatatcccagtcttctgggggggacataggggttcacatggcacacgatgatcagtcagttagctccaaaatagtagctcactgccctccccaggacccgtgcttagtgcatgactgcatagtgtgtgctcatggcctgataaattaccagtgtcacactgctctcagtgcc

SEQ ID NO: 4 - protein, 450 aa, Rift Valley fever virus
  SIGNAL (1)..(18)
MTVLPALAVFALAPVVFAEDPHLRNRPGKGHNYIDGMTQEDATCKPVTYAGACSSFDVLLEKGKFPLFQSYAHHRTLLEAVHDTIIAKADPPSCDLLSAHGNPCMKEKLVMKTHCPNDYQSAHYLNNDGKMASVKCPPKYELTEDCNFCRQMTGASLKKGSYPLQDLFCQSSEDDGSKLKTKMKGVCEVGVQALKKCDGQLSTAHEVVPFAVFKNSKKVYLDKLDLKTEENLLPDSFVCFEHKGQYKGTMDSGQTKRELKSFDISQCPKIGGHGSKKCTGDAAFCSAYECTAQYANAYCSHANGSGIVQIQVSGVWKKPLCVGYERVVVKRELSAKPIQRVEPCTTCITKCEPHGLVVRSTGFKISSAVACASGVCVTGSQSPSTEITLKYPGISQSSGGDIGVHMAHDDQSVSSKIVAHCPPQDPCLVHDCIVCAHGLINYQCHTALSA

SEQ ID NO: 5 - DNA, 1579 bp, Rift Valley fever virus
  Kozak (1)..(4)
  sig_peptide (5)..(58)
caccatgacagtccttccagccttagcagtttttgctttggcacctgttgtttttgcttgttcagaactgattcaggcaagctccagaatcaccacttgctctacagagggtgttaacaccaagtgtagactgtctggcacagcattgatcagagcagggtcagttggggcagaggcttgtttgatgttgaagggggtcaaggaagatcaaaccaagttcttaaagataaaaactgtctcaagtgagctatcatgcagggagggccagagttattggactgggtcctttagccctaaatgtttgagctcaaggagatgccaccttgtcggggaatgccatgtgaataggtgtctgtcttggagggacaatgaaacttcagcagagttttcatttgttggggaaagcacgaccatgcgagagaataagtgttttgagcaatgtggaggatgggggtgtgggtgtttcaatgtgaacccatcttgcttatttgtgcacacgtatctgcagtcagttagaaaagaggcccttagagtttttaactgtatcgactgggtgcataaactcactctagagatcacagactttgatggctctgtttcaacaatagacttgggagcatcatctagccgtttcacaaactggggttcagttagcctctcactggacgcagagggcatttcaggctcaaatagcttttctttcattgagagcccaggcaaagggtatgcaattgttgatgagccattctcagaaattcctcggcaagggttcttgggggagatcaggtgcaattcagagtcctcagtcctgagtgctcatgaatcatgccttagggcaccaaaccttatctcatacaagcccatgatagatcaattggagtgcacaacaaatctgattgatccctttgttgtctttgagaggggttctctgccacagacaaggaatgacaaaacctttgcagcttcaaaaggaaatagaggtgttcaagctttctctaagggctctgtacaagctgatctaactctgatgtttgacaattttgaggtggactttgtgggagcagccgtatcttgtgatgccgccttcttaaatttgacaggttgctattcttgcaatgcaggggccagggtctgcctgtctatcacatccacaggaactggatctctctctgcccacaataaggatgggtctctgcatatagtccttccatcagagaatggaacaaaagaccagtgtcagatactacacttcactgtgcctgaagtagaggaggagtttatgtactcttgtgatggagatgagcggcctctgttggtgaaggggaccctgatagccattgatccatttgatgataggcgggaagcagggggggaatcaacagttgtgaatccaaaatctggatcttggaatttctttgactggttttctggactcatgagttggtttggagggcctcttaaaactatactcctcatttgcctgtatgttgcattatcaattgggctctttttcctccttatatatcttggaagaacaggcctctctaaaatgtggcttgctgccactaagaaggcctca

SEQ ID NO: 6 - protein, 525 aa, Rift Valley fever virus
  SIGNAL (1)..(18)
MTVLPALAVFALAPVVFACSELIQASSRITTCSTEGVNTKCRLSGTALIRAGSVGAEACLMLKGVKEDQTKFLKIKTVSSELSCREGQSYWTGSFSPKCLSSRRCHLVGECHVNRCLSWRDNETSAEFSFVGESTTMRENKCFEQCGGWGCGCFNVNPSCLFVHTYLQSVRKEALRVFNCIDWVHKLTLEITDFDGSVSTIDLGASSSRFTNWGSVSLSLDAEGISGSNSFSFIESPGKGYAIVDEPFSEIPRQGFLGEIRCNSESSVLSAHESCLRAPNLISYKPMIDQLECTTNLIDPFVVFERGSLPQTRNDKTFAASKGNRGVQAFSKGSVQADLTLMFDNFEVDFVGAAVSCDAAFLNLTGCYSCNAGARVCLSITSTGTGSLSAHNKDGSLHIVLPSENGTKDQCQILHFTVPEVEEEFMYSCDGDERPLLVKGTLIAIDPFDDRREAGGESTVVNPKSGSWNFFDWFSGLMSWFGGPLKTILLICLYVALSIGLFFLLIYLGRTGLSKMWLAATKKAS

SEQ ID NO: 7 - DNA, 315 bp, Rift Valley fever virus
  misc_structure (1)..(57): Transmembrane Domain
  misc_structure (58)..(315): Cytosolic Domain
tttgttgttgtgtttgtattcagttctattgcaataatttgtttagctattctttatagggtgcttaagtgcctgaagattgccccaaggaaagttctgaatccactaatgtggatcacagccttcatcagatggatatataagaagatggttgccagagtggcagacaacattaatcaagtgaacagggaaataggatggatggaaggaggtcagttggttctagggaaccctgcccctattcctcgtcatgccccaatcccacgttatagcacatacctgatgttattattgattgtctcatatgcatcagca

SEQ ID NO: 8 - protein, 244 aa, Rift Valley fever virus
  mat_peptide (1)..(244): N Protein
MDNYQELAIQFAAQAVDRNEIEQWVREFAYQGFDARRVIELLKQYGGADWEKDAKKMIVLALTRGNKPRRMMMKMSKEGKATVEALINKYKLKEGNPSRDELTLSRVAAALAGWTCQALVVLSEWLPVTGTTMDGLSPAYPRHMMHPSFAGMVDPSLPGDYLRAILDAHSLYLLQFSRVINPNLRGRTKEEVAATFTQPMNAAVNSNFISHEKRREFLKAFGLVDSNGPSAAVMAAAQAYKTAA

SEQ ID NO: 9 - protein, 265 aa, Rift Valley fever virus
  mat_peptide (1)..(265): NSs Protein
MDYFPVISVDLQSGRRVVSVEYFRGDGPPRIPYSMVGPCCVFLMHHRPSHEVRLRFSDFYNVGEFPYRVGLGDFASNVAPPPAKPFQRLIDLIGHMTLSDFTRFPNLKEAISWPLGEPSLAFFDLSSTRVHRNDDIRRDQIATLAMRSCKITNDLEDSFVGLHRMIATEAILRGIDLCLLPGFDLMYEVAHVQCVRLLQAAKEDISNAVVPNSALIVLMEESLMLRSSLPSMMGRNNWIPVIPPIPDVEMESEEESDDDGFVEVD

SEQ ID NO: 10 - protein, 115 aa, Rift Valley fever virus
  mat_peptide (1)..(115): NSm Protein
MIEGAWDSLREEEMPEELSCSISGIREVKTSSQELYRALKAIIAADGLNNITCHGKDPEDKISLIKGPPHKKRVGIVRCERRRDAKQIGRETMAGIAMTVLPALAVFALAPVVFA

SEQ ID NO: 11 - DNA, 32 bp, Artificial Sequence
  Forawrd Primer N cds
caccatggacaactatcaagaccttgcgatcc

SEQ ID NO: 12 - DNA, 25 bp, Artificial Sequence
  Reverse Primer N cds
ggctgctgtcttgtaagcctgagcg

SEQ ID NO: 13 - DNA, 37 bp, Artificial Sequence
  Forward Primer NSs cds
caccatggattactttcctgtgatatctgttgatttg

SEQ ID NO: 14 - DNA, 34 bp, Artificial Sequence
  Reverse Primer NSs cds
atcaacctcaacaaatccatcatcatcactctcc

SEQ ID NO: 15 - DNA, 27 bp, Artificial Sequence
  Forward Primer NSm cds
caccatgattgaaggagcttgggattc

SEQ ID NO: 16 - DNA, 24 bp, Artificial Sequence
  Reverse Primer NSm cds
agcaaaaacaacaggtgccaaagc

SEQ ID NO: 17 - DNA, 26 bp, Artificial Sequence
  Forward Primer Gne or Gc cds
caccatgacagtccttccagccttag

SEQ ID NO: 18 - DNA, 24 bp, Artificial Sequence
  Reverse Primer Gne cds
ggcactgagagcagtgtgacactg

SEQ ID NO: 19 - DNA, 24 bp, Artificial Sequence
  Reverse Primer Gc cds
tgaggccttcttagtggcagcaag

SEQ ID NO: 20 - DNA, 23 bp, Artificial Sequence
  Forward Primer M13 Sequencing Primer
cccagtcacgacgttgtaaaacg

SEQ ID NO: 21 - DNA, 23 bp, Artificial Sequence
  Reverse Primer M13 Sequencing Primer
agcggataacaatttcacacagg